European Patent Specification EP 3 827 082 B1, published May 14, 2025. Title: ICAM-1 APTAMERS, DIAGNOSTIC AND THERAPEUTIC USES THEREOF. Applicant: Bracco Imaging SpA Consiglio Nazionale delle Ricerche. The sequence listing filed with the application follows.

SEQUENCE LISTING (2 sequences)

SEQ ID NO: 1 - RNA, 55 nt, Artificial Sequence
  synthetic aptamer
ucaugauacguugcgugagcaacugcggcgcuaaaguuugguugacuaguacaug

SEQ ID NO: 2 - RNA, 84 nt, Artificial Sequence
  synthetic aptamer
gggaagagaaggacauaugaucaugauacguugcgugagcaacugcggcgcuaaaguuugguugacuaguacaugaccacuuga